European Patent Specification EP 3 690 041 B1, published September 25, 2024. Title: Tim protein-bound carrier, methods for obtaining, removing and detecting extracelluar membrane vesicles and viruses using said carrier, and kit including said carrier. Applicant: FUJIFILM Wako Pure Chemical Corporation Osaka University. The sequence listing filed with the application follows.

SEQUENCE LISTING (34 sequences)

SEQ ID NO: 1 - protein, 114 aa, mouse Tim4
AASEDTIIGFLGQPVTLPCHYLSWSQSRNSMCWGKGSCPNSKCNAELLRTDGTRIISRKSTKYTLLGKVQFGEVSLTISNTNRGDSGVYCCRIEVPGWFNDVKKNVRLELRRAT

SEQ ID NO: 2 - protein, 113 aa, human Tim4
ETVVTEVLGHRVTLPCLYSSWSHNSNSMCWGKDQCPYSGCKEALIRTDGMRVTSRKSAKYRLQGTIPRGDVSLTILNPSESDSGVYCCRIEVPGWFNDVKINVRLNLQRASTT

SEQ ID NO: 3 - protein, 343 aa, mouse Tim4
MSKGLLLLWLVTELWWLYLTPAASEDTIIGFLGQPVTLPCHYLSWSQSRNSMCWGKGSCPNSKCNAELLRTDGTRIISRKSTKYTLLGKVQFGEVSLTISNTNRGDSGVYCCRIEVPGWFNDVKKNVRLELRRATTTKKPTTTTRPTTTPYVTTTTPELLPTTVMTTSVLPTTTPPQTLATTAFSTAVTTCPSTTPGSFSQETTKGSAFTTESETLPASNHSQRSMMTISTDIAVLRPTGSNPGILPSTSQLTTQKTTLTTSESLQKTTKSHQINSRQTILIIACCVGFVLMVLLFLAFLLRGKVTGANCLQRHKRPDNTEDSDSVLNDMSHGRDDEDGIFTL

SEQ ID NO: 4 - protein, 378 aa, human Tim4
MSKEPLILWLMIEFWWLYLTPVTSETVVTEVLGHRVTLPCLYSSWSHNSNSMCWGKDQCPYSGCKEALIRTDGMRVTSRKSAKYRLQGTIPRGDVSLTILNPSESDSGVYCCRIEVPGWFNDVKINVRLNLQRASTTTHRTATTTTRRTTTTSPTTTRQMTTTPAALPTTVVTTPDLTTGTPLQMTTIAVFTTANTCLSLTPSTLPEEATGLLTPEPSKEGPILTAESETVLPSDSWSSVESTSADTVLLTSKESKVWDLPSTSHVSMWKTSDSVSSPQPGASDTAVPEQNKTTKTGQMDGIPMSMKNEMPISQLLMIIAPSLGFVLFALFVAFLLRGKLMETYCSQKHTRLDYIGDSKNVLNDVQHGREDEDGLFTL

SEQ ID NO: 5 - protein, 252 aa, mouse Tim4
AASEDTIIGFLGQPVTLPCHYLSWSQSRNSMCWGKGSCPNSKCNAELLRTDGTRIISRKSTKYTLLGKVQFGEVSLTISNTNRGDSGVYCCRIEVPGWFNDVKKNVRLELRRATTTKKPTTTTRPTTTPYVTTTTPELLPTTVMTTSVLPTTTPPQTLATTAFSTAVTTCPSTTPGSFSQETTKGSAFTTESETLPASNHSQRSMMTISTDIAVLRPTGSNPGILPSTSQLTTQKTTLTTSESLQKTTKSHQ

SEQ ID NO: 6 - protein, 258 aa, mouse Tim4
AASEDTIIGFLGQPVTLPCHYLSWSQSRNSMCWGKGSCPNSKCNAELLRTDGTRIISRKSTKYTLLGKVQFGEVSLTISNTNRGDSGVYCCRIEVPGWFNDVKKNVRLELRRATTTKKPTTTTRPTTTPYVTTTTPELLPTTVMTTSVLPTTTPPQTLATTAFSTAVTTCPSTTPGSFSQETTKGSAFTTESETLPASNHSQRSMMTISTDIAVLRPTGSNPGILPSTSQLTTQKTTLTTSESLQKTTKSHQINSRQT

SEQ ID NO: 7 - protein, 291 aa, human Tim4
ETVVTEVLGHRVTLPCLYSSWSHNSNSMCWGKDQCPYSGCKEALIRTDGMRVTSRKSAKYRLQGTIPRGDVSLTILNPSESDSGVYCCRIEVPGWFNDVKINVRLNLQRASTTTHRTATTTTRRTTTTSPTTTRQMTTTPAALPTTVVTTPDLTTGTPLQMTTIAVFTTANTCLSLTPSTLPEEATGLLTPEPSKEGPILTAESETVLPSDSWSSVESTSADTVLLTSKESKVWDLPSTSHVSMWKTSDSVSSPQPGASDTAVPEQNKTTKTGQMDGIPMSMKNEMPISQL

SEQ ID NO: 8 - protein, 110 aa, mouse Tim1
YVEVKGVVGHPVTLPCTYSTYRGITTTCWGRGQCPSSACQNTLIWTNGHRVTYQKSSRYNLKGHISEGDVSLTIENSVESDSGLYCCRVEIPGWFNDQKVTFSLQVKPEI

SEQ ID NO: 9 - protein, 110 aa, human Tim1
SVKVGGEAGPSVTLPCHYSGAVTSMCWNRGSCSLFTCQNGIVWTNGTHVTYRKDTRYKLLGDLSRRDVSLTIENTAVSDSGVYCCRVEHRGWFNDMKITVSLEIVPPKVT

SEQ ID NO: 10 - protein, 282 aa, mouse Tim1
MNQIQVFISGLILLLPGAVDSYVEVKGVVGHPVTLPCTYSTYRGITTTCWGRGQCPSSACQNTLIWTNGHRVTYQKSSRYNLKGHISEGDVSLTIENSVESDSGLYCCRVEIPGWFNDQKVTFSLQVKPEIPTRPPRRPTTTRPTATGRPTTISTRSTHVPTSTRVSTSTPPTSTHTWTHKPDWNGTVTSSGDTWSNHTEAIPPGKPQKNPTKGFYVGICIAALLLLLLVSTVAITRYILMKRKSASLSVVAFRVSKIEALQNAAVVHSRAEDNIYIVEDRP

SEQ ID NO: 11 - protein, 364 aa, human Tim1
MHPQVVILSLILHLADSVAGSVKVGGEAGPSVTLPCHYSGAVTSMCWNRGSCSLFTCQNGIVWTNGTHVTYRKDTRYKLLGDLSRRDVSLTIENTAVSDSGVYCCRVEHRGWFNDMKITVSLEIVPPKVTTTPIVTTVPTVTTVRTSTTVPTTTTVPMTTVPTTTVPTTMSIPTTTTVLTTMTVSTTTSVPTTTSIPTTTSVPVTTTVSTFVPPMPLPRQNHEPVATSPSSPQPAETHPTTLQGAIRREPTSSPLYSYTTDGNDTVTESSDGLWNNNQTQLFLEHSLLTANTTKGIYAGVCISVLVLLALLGVIIAKKYFFKKEVQQLSVSFSSLQIKALQNAVEKEVQAEDNIYIENSLYATD

SEQ ID NO: 12 - protein, 191 aa, mouse Tim1
YVEVKGVVGHPVTLPCTYSTYRGITTTCWGRGQCPSSACQNTLIWTNGHRVTYQKSSRYNLKGHISEGDVSLTIENSVESDSGLYCCRVEIPGWFNDQKVTFSLQVKPEIPTRPPRRPTTTRPTATGRPTTISTRSTHVPTSTRVSTSTPPTSTHTWTHKPDWNGTVTSSGDTWSNHTEAIPPGKPQKNPT

SEQ ID NO: 13 - protein, 275 aa, human Tim1
SVKVGGEAGPSVTLPCHYSGAVTSMCWNRGSCSLFTCQNGIVWTNGTHVTYRKDTRYKLLGDLSRRDVSLTIENTAVSDSGVYCCRVEHRGWFNDMKITVSLEIVPPKVTTTPIVTTVPTVTTVRTSTTVPTTTTVPMTTVPTTTVPTTMSIPTTTTVLTTMTVSTTTSVPTTTSIPTTTSVPVTTTVSTFVPPMPLPRQNHEPVATSPSSPQPAETHPTTLQGAIRREPTSSPLYSYTTDGNDTVTESSDGLWNNNQTQLFLEHSLLTANTTKG

SEQ ID NO: 14 - protein, 113 aa, mouse Tim3
LENAYVFEVGKNAYLPCSYTLSTPGALVPMCWGKGFCPWSQCTNELLRTDERNVTYQKSSRYQLKGDLNKGDVSLIIKNVTLDDHGTYCCRIQFPGLMNDKKLELKLDIKAAK

SEQ ID NO: 15 - protein, 114 aa, human Tim3
SEVEYRAEVGQNAYLPCFYTPAAPGNLVPVCWGKGACPVFECGNVVLRTDERDVNYWTSRYWLNGDFRKGDVSLTIENVTLADSGIYCCRIQIPGIMNDEKFNLKLVIKPAKVT

SEQ ID NO: 16 - protein, 281 aa, mouse Tim3
MFSGLTLNCVLLLLQLLLARSLENAYVFEVGKNAYLPCSYTLSTPGALVPMCWGKGFCPWSQCTNELLRTDERNVTYQKSSRYQLKGDLNKGDVSLIIKNVTLDDHGTYCCRIQFPGLMNDKKLELKLDIKAAKVTPAQTAHGDSTTASPRTLTTERNGSETQTLVTLHNNNGTKISTWADEIKDSGETIRTAIHIGVGVSAGLTLALIIGVLILKWYSCKKKKLSSLSLITLANLPPGGLANAGAVRIRSEENIYTIEENVYEVENSNEYYCYVNSQQPS

SEQ ID NO: 17 - protein, 301 aa, human Tim3
MFSHLPFDCVLLLLLLLLTRSSEVEYRAEVGQNAYLPCFYTPAAPGNLVPVCWGKGACPVFECGNVVLRTDERDVNYWTSRYWLNGDFRKGDVSLTIENVTLADSGIYCCRIQIPGIMNDEKFNLKLVIKPAKVTPAPTRQRDFTAAFPRMLTTRGHGPAETQTLGSLPDINLTQISTLANELRDSRLANDLRDSGATIRIGIYIGAGICAGLALALIFGALIFKWYSHSKEKIQNLSLISLANLPPSGLANAVAEGIRSEENIYTIEENVYEVEEPNEYYCYVSSRQQPSQPLGCRFAMP

SEQ ID NO: 18 - protein, 168 aa, mouse Tim3
LENAYVFEVGKNAYLPCSYTLSTPGALVPMCWGKGFCPWSQCTNELLRTDERNVTYQKSSRYQLKGDLNKGDVSLIIKNVTLDDHGTYCCRIQFPGLMNDKKLELKLDIKAAKVTPAQTAHGDSTTASPRTLTTERNGSETQTLVTLHNNNGTKISTWADEIKDSGET

SEQ ID NO: 19 - protein, 179 aa, human Tim3
SEVEYRAEVGQNAYLPCFYTPAAPGNLVPVCWGKGACPVFECGNVVLRTDERDVNYWTSRYWLNGDFRKGDVSLTIENVTLADSGIYCCRIQIPGIMNDEKFNLKLVIKPAKVTPAPTRQRDFTAAFPRMLTTRGHGPAETQTLGSLPDINLTQISTLANELRDSRLANDLRDSGATIR

SEQ ID NO: 20 - DNA, 1032 bp, mouse Tim4
atgtccaaggggcttctcctcctctggctggtgacggagctctggtggctttatctgacaccagctgcctcagaggatacaataatagggtttttgggccagccggtgactttgccttgtcattacctctcgtggtcccagagccgcaacagtatgtgctggggcaaaggttcatgtcccaattccaagtgcaatgcagagcttctccgtacagatggaacaagaatcatctccaggaagtcaacaaaatatacacttttggggaaggtccagtttggtgaagtgtccttgaccatctcaaacaccaatcgaggtgacagtggggtgtactgctgccgtatagaggtgcctggctggttcaatgatgtcaagaagaatgtgcgcttggagctgaggagagccacaacaaccaaaaaaccaacaacaaccacccggccaaccaccaccccttatgtgaccaccaccaccccagagctgcttccaacaacagtcatgaccacatctgttctcccaaccaccacaccaccccagacactagccaccactgccttcagtacagcagtgaccacgtgcccctcaacaacacctggctccttctcacaagaaaccacaaaagggtccgccttcactacagaatcagaaactctgcctgcatccaatcactctcaaagaagcatgatgaccatatctacagacatagccgtactcaggcccacaggctctaaccctgggattctcccatccacttcacagctgacgacacagaaaacaacattaacaacaagtgagtctttgcagaagacaactaaatcacatcagatcaacagcagacagaccatcttgatcattgcctgctgtgtgggatttgtgctaatggtgttattgtttctggcgtttctccttcgagggaaagtcacaggagccaactgtttgcagagacacaagaggccagacaacactgaagatagtgacagcgtcctcaatgacatgtcacacgggagggatgatgaagacgggatcttcactctctga

SEQ ID NO: 21 - DNA, 1137 bp, human Tim4
atgtccaaagaacctctcattctctggctgatgattgagttttggtggctttacctgacaccagtcacttcagagactgttgtgacggaggttttgggtcaccgggtgactttgccctgtctgtactcatcctggtctcacaacagcaacagcatgtgctgggggaaagaccagtgcccctactccggttgcaaggaggcgctcatccgcactgatggaatgagggtgacctcaagaaagtcagcaaaatatagacttcaggggactatcccgagaggtgatgtctccttgaccatcttaaaccccagtgaaagtgacagcggtgtgtactgctgccgcatagaagtgcctggctggttcaacgatgtaaagataaacgtgcgcctgaatctacagagagcctcaacaaccacgcacagaacagcaaccaccaccacacgcagaacaacaacaacaagccccaccaccacccgacaaatgacaacaaccccagctgcacttccaacaacagtcgtgaccacacccgatctcacaaccggaacaccactccagatgacaaccattgccgtcttcacaacagcaaacacgtgcctttcactaaccccaagcacccttccggaggaagccacaggtcttctgactcccgagccttctaaggaagggcccatcctcactgcagaatcagaaactgtcctccccagtgattcctggagtagtgttgagtctacttctgctgacactgtcctgctgacatccaaagagtccaaagtttgggatctcccatcaacatcccacgtgtcaatgtggaaaacgagtgattctgtgtcttctcctcagcctggagcatctgatacagcagttcctgagcagaacaaaacaacaaaaacaggacagatggatggaatacccatgtcaatgaagaatgaaatgcccatctcccaactactgatgatcatcgccccctccttgggatttgtgctcttcgcattgtttgtggcgtttctcctgagagggaaactcatggaaacctattgttcgcagaaacacacaaggctagactacattggagatagtaaaaatgtcctcaatgacgtgcagcatggaagggaagacgaagacggcctttttaccctctaa

SEQ ID NO: 22 - DNA, 849 bp, mouse Tim1
atgaatcagattcaagtcttcatttcaggcctcatactgcttctcccaggcgctgtggattcttatgtggaagtaaagggggtggtgggtcaccctgtcacacttccatgtacttactcaacatatcgtggaatcacaacgacatgttggggccgagggcaatgcccatcttctgcttgtcaaaatacacttatttggaccaatggacatcgtgtcacctatcagaagagcagtcggtacaacttaaaggggcatatttcagaaggagatgtgtccttgacgatagagaactctgttgagagtgacagtggtctgtattgttgtcgagtggagattcctggatggtttaatgatcagaaagtgaccttttcattgcaagttaaaccagagattcccacacgtcctccaagaagacccacaactacaaggcccacagctacaggaagacccacgactatttcaacaagatccacacatgtaccaacatcaaccagagtctctacctccactcctccaacatctacacacacatggactcacaaaccagactggaatggcactgtgacatcctcaggagatacctggagtaatcacactgaagcaatccctccagggaagccgcagaaaaaccctactaagggcttctatgttggcatctgcatcgcagccctgctgctactgctccttgtgagcaccgtggctatcaccaggtacatacttatgaaaaggaagtcagcatctctaagcgtggttgccttccgtgtctctaagattgaagctttgcagaacgcagcggttgtgcattcccgagctgaagacaacatctacattgttgaagatagaccttga

SEQ ID NO: 23 - DNA, 1095 bp, human Tim1
atgcatcctcaagtggtcatcttaagcctcatcctacatctggcagattctgtagctggttctgtaaaggttggtggagaggcaggtccatctgtcacactaccctgccactacagtggagctgtcacatccatgtgctggaatagaggctcatgttctctattcacatgccaaaatggcattgtctggaccaatggaacccacgtcacctatcggaaggacacacgctataagctattgggggacctttcaagaagggatgtctctttgaccatagaaaatacagctgtgtctgacagtggcgtatattgttgccgtgttgagcaccgtgggtggttcaatgacatgaaaatcaccgtatcattggagattgtgccacccaaggtcacgactactccaattgtcacaactgttccaaccgtcacgactgttcgaacgagcaccactgttccaacgacaacgactgttccaatgacgactgttccaacgacaactgttccaacaacaatgagcattccaacgacaacgactgttctgacgacaatgactgtttcaacgacaacgagcgttccaacgacaacgagcattccaacaacaacaagtgttccagtgacaacaactgtctctacctttgttcctccaatgcctttgcccaggcagaaccatgaaccagtagccacttcaccatcttcacctcagccagcagaaacccaccctacgacactgcagggagcaataaggagagaacccaccagctcaccattgtactcttacacaacagatgggaatgacaccgtgacagagtcttcagatggcctttggaataacaatcaaactcaactgttcctagaacatagtctactgacggccaataccactaaaggaatctatgctggagtctgtatttctgtcttggtgcttcttgctcttttgggtgtcatcattgccaaaaagtatttcttcaaaaaggaggttcaacaactaagtgtttcatttagcagccttcaaattaaagctttgcaaaatgcagttgaaaaggaagtccaagcagaagacaatatctacattgagaatagtctttatgccacggactaa

SEQ ID NO: 24 - DNA, 846 bp, mouse Tim3
atgttttcaggtcttaccctcaactgtgtcctgctgctgctgcaactactacttgcaaggtcattggaaaatgcttatgtgtttgaggttggtaagaatgcctatctgccctgcagttacactctatctacacctggggcacttgtgcctatgtgctggggcaagggattctgtccttggtcacagtgtaccaacgagttgctcagaactgatgaaagaaatgtgacatatcagaaatccagcagataccagctaaagggcgatctcaacaaaggagacgtgtctctgatcataaagaatgtgactctggatgaccatgggacctactgctgcaggatacagttccctggtcttatgaatgataaaaaattagaactgaaattagacatcaaagcagccaaggtcactccagctcagactgcccatggggactctactacagcttctccaagaaccctaaccacggagagaaatggttcagagacacagacactggtgaccctccataataacaatggaacaaaaatttccacatgggctgatgaaattaaggactctggagaaacgatcagaactgctatccacattggagtgggagtctctgctgggttgaccctggcacttatcattggtgtcttaatccttaaatggtattcctgtaagaaaaagaagttatcgagtttgagccttattacactggccaacttgcctccaggagggttggcaaatgcaggagcagtcaggattcgctctgaggaaaatatctacaccatcgaggagaacgtatatgaagtggagaattcaaatgagtactactgctacgtcaacagccagcagccatcctga

SEQ ID NO: 25 - DNA, 906 bp, human Tim3
atgttttcacatcttccctttgactgtgtcctgctgctgctgctgctactacttacaaggtcctcagaagtggaatacagagcggaggtcggtcagaatgcctatctgccctgcttctacaccccagccgccccagggaacctcgtgcccgtctgctggggcaaaggagcctgtcctgtgtttgaatgtggcaacgtggtgctcaggactgatgaaagggatgtgaattattggacatccagatactggctaaatggggatttccgcaaaggagatgtgtccctgaccatagagaatgtgactctagcagacagtgggatctactgctgccggatccaaatcccaggcataatgaatgatgaaaaatttaacctgaagttggtcatcaaaccagccaaggtcacccctgcaccgactcggcagagagacttcactgcagcctttccaaggatgcttaccaccaggggacatggcccagcagagacacagacactggggagcctccctgatataaatctaacacaaatatccacattggccaatgagttacgggactctagattggccaatgacttacgggactctggagcaaccatcagaataggcatctacatcggagcagggatctgtgctgggctggctctggctcttatcttcggcgctttaattttcaaatggtattctcatagcaaagagaagatacagaatttaagcctcatctctttggccaacctccctccctcaggattggcaaatgcagtagcagagggaattcgctcagaagaaaacatctataccattgaagagaacgtatatgaagtggaggagcccaatgagtattattgctatgtcagcagcaggcagcaaccctcacaacctttgggttgtcgctttgcaatgccatag

SEQ ID NO: 26 - DNA, 822 bp, mouse Tim4
atgtccaaggggcttctcctcctctggctggtgacggagctctggtggctttatctgacaccagctgcctcagaggatacaataatagggtttttgggccagccggtgactttgccttgtcattacctctcgtggtcccagagccgcaacagtatgtgctggggcaaaggttcatgtcccaattccaagtgcaatgcagagcttctccgtacagatggaacaagaatcatctccaggaagtcaacaaaatatacacttttggggaaggtccagtttggtgaagtgtccttgaccatctcaaacaccaatcgaggtgacagtggggtgtactgctgccgtatagaggtgcctggctggttcaatgatgtcaagaagaatgtgcgcttggagctgaggagagccacaacaaccaaaaaaccaacaacaaccacccggccaaccaccaccccttatgtgaccaccaccaccccagagctgcttccaacaacagtcatgaccacatctgttctcccaaccaccacaccaccccagacactagccaccactgccttcagtacagcagtgaccacgtgcccctcaacaacacctggctccttctcacaagaaaccacaaaagggtccgccttcactacagaatcagaaactctgcctgcatccaatcactctcaaagaagcatgatgaccatatctacagacatagccgtactcaggcccacaggctctaaccctgggattctcccatccacttcacagctgacgacacagaaaacaacattaacaacaagtgagtctttgcagaagacaactaaatcacatcagtga

SEQ ID NO: 27 - DNA, 840 bp, mouse Tim4
atgtccaaggggcttctcctcctctggctggtgacggagctctggtggctttatctgacaccagctgcctcagaggatacaataatagggtttttgggccagccggtgactttgccttgtcattacctctcgtggtcccagagccgcaacagtatgtgctggggcaaaggttcatgtcccaattccaagtgcaatgcagagcttctccgtacagatggaacaagaatcatctccaggaagtcaacaaaatatacacttttggggaaggtccagtttggtgaagtgtccttgaccatctcaaacaccaatcgaggtgacagtggggtgtactgctgccgtatagaggtgcctggctggttcaatgatgtcaagaagaatgtgcgcttggagctgaggagagccacaacaaccaaaaaaccaacaacaaccacccggccaaccaccaccccttatgtgaccaccaccaccccagagctgcttccaacaacagtcatgaccacatctgttctcccaaccaccacaccaccccagacactagccaccactgccttcagtacagcagtgaccacgtgcccctcaacaacacctggctccttctcacaagaaaccacaaaagggtccgccttcactacagaatcagaaactctgcctgcatccaatcactctcaaagaagcatgatgaccatatctacagacatagccgtactcaggcccacaggctctaaccctgggattctcccatccacttcacagctgacgacacagaaaacaacattaacaacaagtgagtctttgcagaagacaactaaatcacatcagatcaacagcagacagacctga

SEQ ID NO: 28 - DNA, 948 bp, human Tim4
atgtccaaagaacctctcattctctggctgatgattgagttttggtggctttacctgacaccagtcacttcagagactgttgtgacggaggttttgggtcaccgggtgactttgccctgtctgtactcatcctggtctcacaacagcaacagcatgtgctgggggaaagaccagtgcccctactccggttgcaaggaggcgctcatccgcactgatggaatgagggtgacctcaagaaagtcagcaaaatatagacttcaggggactatcccgagaggtgatgtctccttgaccatcttaaaccccagtgaaagtgacagcggtgtgtactgctgccgcatagaagtgcctggctggttcaacgatgtaaagataaacgtgcgcctgaatctacagagagcctcaacaaccacgcacagaacagcaaccaccaccacacgcagaacaacaacaacaagccccaccaccacccgacaaatgacaacaaccccagctgcacttccaacaacagtcgtgaccacacccgatctcacaaccggaacaccactccagatgacaaccattgccgtcttcacaacagcaaacacgtgcctttcactaaccccaagcacccttccggaggaagccacaggtcttctgactcccgagccttctaaggaagggcccatcctcactgcagaatcagaaactgtcctccccagtgattcctggagtagtgttgagtctacttctgctgacactgtcctgctgacatccaaagagtccaaagtttgggatctcccatcaacatcccacgtgtcaatgtggaaaacgagtgattctgtgtcttctcctcagcctggagcatctgatacagcagttcctgagcagaacaaaacaacaaaaacaggacagatggatggaatacccatgtcaatgaagaatgaaatgcccatctcccaactatga

SEQ ID NO: 29 - DNA, 639 bp, mouse Tim1
atgaatcagattcaagtcttcatttcaggcctcatactgcttctcccaggcgctgtggattcttatgtggaagtaaagggggtggtgggtcaccctgtcacacttccatgtacttactcaacatatcgtggaatcacaacgacatgttggggccgagggcaatgcccatcttctgcttgtcaaaatacacttatttggaccaatggacatcgtgtcacctatcagaagagcagtcggtacaacttaaaggggcatatttcagaaggagatgtgtccttgacgatagagaactctgttgagagtgacagtggtctgtattgttgtcgagtggagattcctggatggtttaatgatcagaaagtgaccttttcattgcaagttaaaccagagattcccacacgtcctccaagaagacccacaactacaaggcccacagctacaggaagacccacgactatttcaacaagatccacacatgtaccaacatcaaccagagtctctacctccactcctccaacatctacacacacatggactcacaaaccagactggaatggcactgtgacatcctcaggagatacctggagtaatcacactgaagcaatccctccagggaagccgcagaaaaaccctacttga

SEQ ID NO: 30 - DNA, 888 bp, human Tim1
atgcatcctcaagtggtcatcttaagcctcatcctacatctggcagattctgtagctggttctgtaaaggttggtggagaggcaggtccatctgtcacactaccctgccactacagtggagctgtcacatccatgtgctggaatagaggctcatgttctctattcacatgccaaaatggcattgtctggaccaatggaacccacgtcacctatcggaaggacacacgctataagctattgggggacctttcaagaagggatgtctctttgaccatagaaaatacagctgtgtctgacagtggcgtatattgttgccgtgttgagcaccgtgggtggttcaatgacatgaaaatcaccgtatcattggagattgtgccacccaaggtcacgactactccaattgtcacaactgttccaaccgtcacgactgttcgaacgagcaccactgttccaacgacaacgactgttccaatgacgactgttccaacgacaactgttccaacaacaatgagcattccaacgacaacgactgttctgacgacaatgactgtttcaacgacaacgagcgttccaacgacaacgagcattccaacaacaacaagtgttccagtgacaacaactgtctctacctttgttcctccaatgcctttgcccaggcagaaccatgaaccagtagccacttcaccatcttcacctcagccagcagaaacccaccctacgacactgcagggagcaataaggagagaacccaccagctcaccattgtactcttacacaacagatgggaatgacaccgtgacagagtcttcagatggcctttggaataacaatcaaactcaactgttcctagaacatagtctactgacggccaataccactaaaggatga

SEQ ID NO: 31 - DNA, 570 bp, mouse Tim3
atgttttcaggtcttaccctcaactgtgtcctgctgctgctgcaactactacttgcaaggtcattggaaaatgcttatgtgtttgaggttggtaagaatgcctatctgccctgcagttacactctatctacacctggggcacttgtgcctatgtgctggggcaagggattctgtccttggtcacagtgtaccaacgagttgctcagaactgatgaaagaaatgtgacatatcagaaatccagcagataccagctaaagggcgatctcaacaaaggagacgtgtctctgatcataaagaatgtgactctggatgaccatgggacctactgctgcaggatacagttccctggtcttatgaatgataaaaaattagaactgaaattagacatcaaagcagccaaggtcactccagctcagactgcccatggggactctactacagcttctccaagaaccctaaccacggagagaaatggttcagagacacagacactggtgaccctccataataacaatggaacaaaaatttccacatgggctgatgaaattaaggactctggagaaacgtga

SEQ ID NO: 32 - DNA, 603 bp, human Tim3
atgttttcacatcttccctttgactgtgtcctgctgctgctgctgctactacttacaaggtcctcagaagtggaatacagagcggaggtcggtcagaatgcctatctgccctgcttctacaccccagccgccccagggaacctcgtgcccgtctgctggggcaaaggagcctgtcctgtgtttgaatgtggcaacgtggtgctcaggactgatgaaagggatgtgaattattggacatccagatactggctaaatggggatttccgcaaaggagatgtgtccctgaccatagagaatgtgactctagcagacagtgggatctactgctgccggatccaaatcccaggcataatgaatgatgaaaaatttaacctgaagttggtcatcaaaccagccaaggtcacccctgcaccgactcggcagagagacttcactgcagcctttccaaggatgcttaccaccaggggacatggcccagcagagacacagacactggggagcctccctgatataaatctaacacaaatatccacattggccaatgagttacgggactctagattggccaatgacttacgggactctggagcaaccatcagatga

SEQ ID NO: 33 - DNA, 846 bp, mouse Tim4
  FLAG tag (820)..(843)
atgtccaaggggcttctcctcctctggctggtgacggagctctggtggctttatctgacaccagctgcctcagaggatacaataatagggtttttgggccagccggtgactttgccttgtcattacctctcgtggtcccagagccgcaacagtatgtgctggggcaaaggttcatgtcccaattccaagtgcaatgcagagcttctccgtacagatggaacaagaatcatctccaggaagtcaacaaaatatacacttttggggaaggtccagtttggtgaagtgtccttgaccatctcaaacaccaatcgaggtgacagtggggtgtactgctgccgtatagaggtgcctggctggttcaatgatgtcaagaagaatgtgcgcttggagctgaggagagccacaacaaccaaaaaaccaacaacaaccacccggccaaccaccaccccttatgtgaccaccaccaccccagagctgcttccaacaacagtcatgaccacatctgttctcccaaccaccacaccaccccagacactagccaccactgccttcagtacagcagtgaccacgtgcccctcaacaacacctggctccttctcacaagaaaccacaaaagggtccgccttcactacagaatcagaaactctgcctgcatccaatcactctcaaagaagcatgatgaccatatctacagacatagccgtactcaggcccacaggctctaaccctgggattctcccatccacttcacagctgacgacacagaaaacaacattaacaacaagtgagtctttgcagaagacaactaaatcacatcaggattacaaggatgacgacgataagtaa

SEQ ID NO: 34 - DNA, 840 bp, mouse Tim4
  His tag (820)..(837)
atgtccaaggggcttctcctcctctggctggtgacggagctctggtggctttatctgacaccagctgcctcagaggatacaataatagggtttttgggccagccggtgactttgccttgtcattacctctcgtggtcccagagccgcaacagtatgtgctggggcaaaggttcatgtcccaattccaagtgcaatgcagagcttctccgtacagatggaacaagaatcatctccaggaagtcaacaaaatatacacttttggggaaggtccagtttggtgaagtgtccttgaccatctcaaacaccaatcgaggtgacagtggggtgtactgctgccgtatagaggtgcctggctggttcaatgatgtcaagaagaatgtgcgcttggagctgaggagagccacaacaaccaaaaaaccaacaacaaccacccggccaaccaccaccccttatgtgaccaccaccaccccagagctgcttccaacaacagtcatgaccacatctgttctcccaaccaccacaccaccccagacactagccaccactgccttcagtacagcagtgaccacgtgcccctcaacaacacctggctccttctcacaagaaaccacaaaagggtccgccttcactacagaatcagaaactctgcctgcatccaatcactctcaaagaagcatgatgaccatatctacagacatagccgtactcaggcccacaggctctaaccctgggattctcccatccacttcacagctgacgacacagaaaacaacattaacaacaagtgagtctttgcagaagacaactaaatcacatcagcatcatcatcatcatcattga